European Patent Specification EP 3 903 772 B1, published August 6, 2025. Title: COMPOSITIONS AND METHODS TO PROMOTE BONE FORMATION. Applicant: Research Foundation of State University of New York. Application not yet assigned. The sequence listing filed with the application follows.

SEQUENCE LISTING (5 sequences)

SEQ ID NO: 1 - protein, 5 aa, Artificial Sequence
  Synthetic Peptide
YGGFM

SEQ ID NO: 2 - protein, 5 aa, Artificial Sequence
  Synthetic Peptide
YGGFL

SEQ ID NO: 3 - protein, 6 aa, Artificial Sequence
  Synthetic Peptide
  MISC_FEATURE (1)..(1): Xaa is N, N-diallyl-Tyrosine
  MISC_FEATURE (3)..(4): Xaa is Aib (aminoisobutytic acid)
  L (6)..(6): Leu is Leu-OH
XYXXFL

SEQ ID NO: 4 - protein, 8 aa, Artificial Sequence
  Synthetic Peptide
  F (1)..(1): Phe at position 1 is D-Phe
  MISC_FEATURE (7)..(7): Xaa is Pen (Pencillamine)
  T (8)..(8): Thr is Thr-NH2
FCYWKTXT

SEQ ID NO: 5 - protein, 50 aa, Artificial Sequence
  Synthetic Peptide
QSALDYFMFAVRCRHQRRQLVHFAWEHFRPRCKFVWGPQDKLRRFKPSSL